European Patent Application EP 4 166 657 A1, published April 19, 2023. Title: Recombinant Herpes Simplex Virus Containing Expression Cassette Expressing a Fused Protein of Tumor Cell-targeting Domain and Extracellular Damain of HVEM and Use of the Same. Applicant: KOREA, gencellmed. The sequence listing filed with the application follows.

SEQUENCE LISTING (36 sequences)

SEQ ID NO: 1 - protein, 838 aa, Artificial Sequence
  gH
MGNGLWFVGVILLGVAWGQVHDWTEQTDPWFLDGLGMDRMYWRDTNTGRLWLPNTPDPQKPPRGFLAPPDELNLTTASLPLLRWYEERFCFVLVTTAEFPRDPGQLLYISKTYLLGRPPNASLPAPITVEPTAQPPPAVAPLKGLLHNPTASVLLRSRAWVTFSAVPDPEALTFPRGDNVATASHPSGPRDTPPPRPPVGARRHPTTELDITHLHNASTTWLATRGLLRSPGRYVYFSPSASTWPVGIWTTGELVLGCDAALVRARYGREFMGLVISMHDSPPVEVMVVPAGQTLDRVGDPADENPPGALPGPPGGPRYRVFVLGSLTRADNGSALDALRRVGGYPEEGTNYAQFLSRAYAEFFSGDAGAEQGPRPPLFWRLTGLLATSGFAFVNAAHANGAVCLSDLLGFLAHSRALAGLAARGAAGCAADSVFFNVSVLDPTARLQLEARLQHLVAEILEREQSLALHALGYQLAFVLDSPSAYDAVAPSAAHLIDALYAEFLGGRVLTTPVVHRALFYASAVLRQPFLAGVPSAVQRERARRSLLIASALCTSDVAAATNADLRTALARADHQKTLFWLPDHFSPCAASLRFDLDESVFILDALAQATRSETPVEVLAQQTHGLASTLTRWAHYNALIRAFVPEASHRCGGQSANVEPRILVPITHNASYVVTHSPLPRGIGYKLTGVDVRRPLFLTYLTATCEGSTRDIESKRLVRTQNQRDLGLVGAVFMRYTPAGEVMSVLLVDTDNTQQQIAAGPTEGAPSVFSSDVPSTALLLFPNGTVIHLLAFDTQPVAAIAPGFLAASALGVVMITAALAGILKVLRTSVPFFWRRE

SEQ ID NO: 2 - protein, 904 aa, Artificial Sequence
  gB
MHQGAPSWGRRWFVVWALLGLTLGVLVASAAPSSPGTPGVAAATQAANGGPATPAPPALGAAPTGDPKPKKNKKPKNPTPPRPAGDNATVAAGHATLREHLRDIKAENTDANFYVCPPPTGATVVQFEQPRRCPTRPEGQNYTEGIAVVFKENIAPYKFKATMYYKDVTVSQVWFGHRYSQFMGIFEDRAPVPFEEVIDKINAKGVCRSTAKYVRNNLETTAFHRDDHETDMELKPANAATRTSRGWHTTDLKYNPSRVEAFHRYGTTVNCIVEEVDARSVYPYDEFVLATGDFVYMSPFYGYREGSHTEHTSYTADRFKQVDGFYARDLTTKARATAPTTRNLLTTPKFTVAWDWVPKRPSVCTMTKWQEVDEMLRSEYGGSFRFSSDAISTTFTTNLTEYPLSRVDLGDCIGKDARDAMDRIFARRYNATHIKVGQPQYYLANGGFLIAYQPLLSNTLAELYVREHLREQSRKPPNPTPPPPGASANASVERIKTTSSIEFARLQFTYNHIQRHVNDMLGRVAIAWCELQNHELTLWNEARKLNPNAIASVTVGRRVSARMLGDVMAVSTCVPVAADNVIVQNSMRISSRPGACYSRPLVSFRYEDQGPLVEGQLGENNELRLTRDAIEPCTVGHRRYFTFGGGYVYFEEYAYSHQLSRADITTVSTFIDLNITMLEDHEFVPLEVYTRHEIKDSGLLDYTEVQRRNQLHDLRFADIDTVIHADANAAMFAGLGAFFEGMGDLGRAVGKVVMGIVGGVVSAVSGVSSFMSNPFGALAVGLLVLAGLAAAFFAFRYVMRLQSNPMKALYPLTTKELKNPTNPDASGEGEEGGDFDEAKLAEAREMIRYMALVSAMERTEHKAKKKGTSALLSAKVTDMVMRKRRNTNYTQVPNKDGDADEDDL

SEQ ID NO: 3 - protein, 511 aa, Artificial Sequence
  gC
MAPGRVGLAVVLWSLLWLGAGVAGGSETASTGPTITAGAVTNASEAPTSGSPGSAASPEVTPTSTPNPNNVTQNKTTPTEPASPPTTPKPTSTPKSPPTSTPDPKPKNNTTPAKSGRPTKPPGPVWCDRRDPLARYGSRVQIRCRFRNSTRMEFRLQIWRYSMGPSPPIAPAPDLEEVLTNITAPPGGLLVYDSAPNLTDPHVLWAEGAGPGADPPLYSVTGPLPTQRLIIGEVTPATQGMYYLAWGRMDSPHEYGTWVRVRMFRPPSLTLQPHAVMEGQPFKATCTAAAYYPRNPVEFVWFEDDRQVFNPGQIDTQTHEHPDGFTTVSTVTSEAVGGQVPPRTFTCQMTWHRDSVMFSRRNATGLALVLPRPTITMEFGVRHVVCTAGCVPEGVTFAWFLGDDPSPAAKSAVTAQESCDHPGLATVRSTLPISYDYSEYICRLTGYPAGIPVLEHHGSHQPPPRDPTERQVIEAIEWVGIGIGVLAAGVLVVTAIVYVVRTSQSRQRHRR

SEQ ID NO: 4 - protein, 120 aa, Artificial Sequence [sequence omitted]

SEQ ID NO: 5 - protein, 107 aa, Artificial Sequence [sequence omitted]

SEQ ID NO: 6 - protein, 113 aa, Artificial Sequence
  EpCAM VL
DIQMTQSPSSLSASVGDRVTITCRSTKSLLHSNGITYLYWYQQKPGKAPKLLIYQMSNLASGVPSRFSSSGSGTDFTLTISSLQPEDFATYYCAQNLEIPRTFGQGTKVELKR

SEQ ID NO: 7 - protein, 838 aa, Artificial Sequence; identical to SEQ ID NO: 1
  EpCAM VH

SEQ ID NO: 8 - protein, 106 aa, Artificial Sequence
  CEA VL
DIQMTQSPASLSASVGDTVTITCRASENIYSYLAWYQQKQGKSPQLLVYAKALSEGVPSRFSGSGSGTQFSLRINSLQPEDFGDYYCQHHYNSPYTFGGGTKLEIK

SEQ ID NO: 9 - protein, 115 aa, Artificial Sequence
  CEA VH
QIQLVQSGELKKPGETVKISCKASGYSFTNDGINWVKQAPGKGFKYMGWINTITGEPTYTEDFKGRFAFSLETSASTAYLQINNLKDEDTATFFCAKGTGTSAYWGQGTLVTVSA

SEQ ID NO: 10 - protein, 369 aa, Artificial Sequence
  gD
KYALADASLKMADPNRFRGKDLPVLDQLTDPPGVRRVYHIQAGLPDPFQPPSLPITVYYAVLERACRSVLLNAPSEAPQIVRGASEDVRKQPYNLTIAWFRMGGNCAIPITVMEYTECSYNKSLGACPIRTQPRWNYYDSFSAVSEDNLGFLMHAPAFETAGTYLRLVKINDWTEITQFILEHRAKGSCKYALPLRIPPSACLSPQAYQQGVTVDSIGMLPRFIPENQRTVAVYSLKIAGWHGPKAPYTSTLLPPELSETPNATQPELAPEDPEDSALLEDPVGTVAPQIPPNWHIPSIQDAATPYHPPATPNNMGLIAGAVGGSLLAALVICGIVYWMHRRTRKAPKRIRLPHIREDDQPSSHQPLFY

SEQ ID NO: 11 - DNA, 60 bp, Artificial Sequence
  gD-rpsL For
cccaggcctaccagcagggggtgacggtggacagcatcgggatgctgcccggcctggtga

SEQ ID NO: 12 - DNA, 88 bp, Artificial Sequence
  gD-rpsL Rev
ccggcgatcttcaagctgtatacggcgacggtgcgctggttctcggggattcagaagaactcgtcaagaaggcgtgatggcgggatcg

SEQ ID NO: 13 - DNA, 106 bp, Artificial Sequence
  gD R222N_F223I_mutant
cccaggcctaccagcagggggtgacggtggacagcatcgggatgctgcccaatatcatccccgagaaccagcgcaccgtcgccgtatacagcttgaagatcgccgg

SEQ ID NO: 14 - DNA, 74 bp, Artificial Sequence
  UL26/27-rpsL_For
gcgtgggggggaggaaatcggcactgaccaagggggtccgttttgtcacgtcagaagaactcgtcaagaaggcg

SEQ ID NO: 15 - DNA, 74 bp, Artificial Sequence
  UL26/27-rpsL_Rev
aacacataaactcccccgggtgtccgcggcctgtttcctctttcctttccggcctggtgatgatggcgggatcg

SEQ ID NO: 16 - DNA, 74 bp, Artificial Sequence
  UL26-tkpA_For
gcgtgggggggaggaaatcggcactgaccaagggggtccgttttgtcacggcctcagaagccatagagcccacc

SEQ ID NO: 17 - DNA, 74 bp, Artificial Sequence
  UL27-pCMV_Rev
aacacataaactcccccgggtgtccgcggcctgtttcctctttcctttcctatacgcgttgacattgattattg

SEQ ID NO: 18 - protein, 15 aa, Artificial Sequence
  HER2 Linker
GGGGSGGGGSGGGGS

SEQ ID NO: 19 - protein, 13 aa, Artificial Sequence
  HER2scFv C-terminus Linker
AAASSGGGSGSGG

SEQ ID NO: 20 - protein, 12 aa, Artificial Sequence
  HER2scFv N-terminus Linker
SGGGSGSGGAAA

SEQ ID NO: 21 - protein, 27 aa, Artificial Sequence
  EpCAM Linker
ATPSHNSHQVPSAGGPTANSGTSGSEV

SEQ ID NO: 22 - protein, 12 aa, Artificial Sequence
  EpCAMscFv N-terminus
AAASSGGGSGSG

SEQ ID NO: 23 - protein, 14 aa, Artificial Sequence
  EpCAMscFv C-terminus
SSGGGSGSGGSAAA

SEQ ID NO: 24 - protein, 17 aa, Artificial Sequence
  CEA Linker
SSGGGGSGGGGSGGGGS

SEQ ID NO: 25 - protein, 13 aa, Artificial Sequence
  CEAscFv N-terminus Linker
AAASSGGGSGSGG

SEQ ID NO: 26 - protein, 12 aa, Artificial Sequence
  CEAscFv C-terminus Linker
SSGGGSGSGAAA

SEQ ID NO: 27 - protein, 268 aa, Artificial Sequence
  HER2scFv ligand whole sequence
AAASSGGGSGSGGEVQLVESGGGLVQPGGSLRLSCAASGFNIKDTYIHWVRQAPGKGLEWVARIYPTNGYTRYADSVKGRFTISADTSKNTAYLQMNSLRAEDTAVYYCSRWGGDGFYAMDYWGQGTLVTVSSGGGGSGGGGSGGGGSDIQMTQSPSSLSASVGDRVTITCRASQDVNTAVAWYQQKPGKAPKLLIYSASFLYSGVPSRFSGSRSGTDFTLTISSLQPEDFATYYCQQHYTTPPTFGQGTKVEIKSGGGSGSGGSAAA

SEQ ID NO: 28 - DNA, 801 bp, Artificial Sequence
  HER2scFv ligand whole sequence
gcggccgccagtagtggcggtggctctggttccggtggagaggtgcagctggttgaatctggcggaggactggttcagcctggcggatctctgagactgtcttgtgccgccagcggcttcaacatcaaggacacctacatccactgggtccgacaggcccctggcaaaggacttgaatgggtcgccagaatctaccccaccaacggctacaccagatacgccgactctgtgaagggcagattcaccatcagcgccgacaccagcaagaacaccgcctacctgcagatgaacagcctgagagccgaggacaccgccgtgtactactgttctagatggggaggcgacggcttctacgccatggattattggggccagggcaccctggtcacagtttctagcggaggcggaggttctggcggcggaggaagtggtggcggaggctctgatatccagatgacacagagccccagcagcctgtctgcctctgtgggagacagagtgaccatcacctgtagagccagccaggacgtgaacacagccgtggcttggtatcagcagaagcctggcaaggcccctaagctgctgatctacagcgccagctttctgtacagcggcgtgcccagcagattcagcggctctagaagcggcaccgacttcaccctgaccataagcagtctgcagcccgaggacttcgccacctactactgtcagcagcactacaccacacctccaaccttcggacagggcaccaaggtggaaatcaagggtggaggctctggttccggtggatccgcggccgcg

SEQ ID NO: 29 - protein, 280 aa, Artificial Sequence
  EpCAMscFv ligand whole sequence
AAASSGGGSGSGDIQMTQSPSSLSASVGDRVTITCRSTKSLLHSNGITYLYWYQQKPGKAPKLLIYQMSNLASGVPSRFSSSGSGTDFTLTISSLQPEDFATYYCAQNLEIPRTFGQGTKVELKRATPSHNSHQVPSAGGPTANSGTSGSEVQLVQSGPGLVQPGGSVRISCAASGYTFTNYGMNWVKQAPGKGLEWMGWINTYTGESTYADSFKGRFTFSLDTSASAAYLQINSLRAEDTAVYYCARFAIKGDYWGQGTLLTVSSSSGGGSGSGGSAAA

SEQ ID NO: 30 - DNA, 840 bp, Artificial Sequence
  EpCAMscFv ligand whole sequence
gcggccgccagtagtggcggtggctctggttccggtgatatccagatgacccagtccccgtcctccctgagtgcttctgttggtgaccgtgttaccatcacctgccgttccaccaaatccctcctgcactccaacggtatcacctacctttattggtatcaacagaaaccgggtaaagctccgaaacttctgatctaccagatgtccaacctggcttccggtgttccgtctcgtttctccagttctggttctggtaccgacttcaccctgaccatctcttctctgcagccggaagacttcgctacctactactgcgctcagaacctggaaatcccgcgtaccttcggtcagggtaccaaagttgaacttaagcgcgctaccccgtctcacaactcccaccaggttccatccgcaggcggtccgactgctaactctggaactagtggatccgaagtacagctggttcagtccggcccgggtcttgttcaaccgggtggttccgttcgtatctcttgcgctgcttctggttacacgttcaccaactacggcatgaactgggtcaaacaggctccgggtaaaggcctggaatggatgggctggatcaacacctacaccggtgaatccacctacgctgactccttcaaaggtcgcttcactttctccctcgacacaagtgctagtgctgcatacctccaaatcaactcgctgcgtgcagaggatacagcagtctattactgcgcccgtttcgctatcaaaggtgactactggggtcaaggcacgctgctgaccgtttcctcgtcttccggtggaggctctggttccggtggatccgcggccgcg

SEQ ID NO: 31 - protein, 262 aa, Artificial Sequence
  CEAscFv ligand whole sequence
AAASSGGGSGSGGDIQMTQSPASLSASVGDTVTITCRASENIYSYLAWYQQKQGKSPQLLVYAKALSEGVPSRFSGSGSGTQFSLRINSLQPEDFGDYYCQHHYNSPYTFGGGTKLEIKSSGGGGSGGGGSGGGGSQIQLVQSGELKKPGETVKISCKASGYSFTNDGINWVKQAPGKGFKYMGWINTITGEPTYTEDFKGRFAFSLETSASTAYLQINNLKDEDTATFFCAKGTGTSAYWGQTLVTVSASSGGGSGSGAAA

SEQ ID NO: 32 - DNA, 801 bp, Artificial Sequence
  CEAscFv ligand whole sequence
gcggccgccagtagtggcggtggctctggttccggtggagaggtgcagctggttgaatctggcggaggactggttcagcctggcggatctctgagactgtcttgtgccgccagcggcttcaacatcaaggacacctacatccactgggtccgacaggcccctggcaaaggacttgaatgggtcgccagaatctaccccaccaacggctacaccagatacgccgactctgtgaagggcagattcaccatcagcgccgacaccagcaagaacaccgcctacctgcagatgaacagcctgagagccgaggacaccgccgtgtactactgttctagatggggaggcgacggcttctacgccatggattattggggccagggcaccctggtcacagtttctagcggaggcggaggttctggcggcggaggaagtggtggcggaggctctgatatccagatgacacagagccccagcagcctgtctgcctctgtgggagacagagtgaccatcacctgtagagccagccaggacgtgaacacagccgtggcttggtatcagcagaagcctggcaaggcccctaagctgctgatctacagcgccagctttctgtacagcggcgtgcccagcagattcagcggctctagaagcggcaccgacttcaccctgaccataagcagtctgcagcccgaggacttcgccacctactactgtcagcagcactacaccacacctccaaccttcggacagggcaccaaggtggaaatcaagtcttccggtggaggctctggttccggtgcggccgcg

SEQ ID NO: 33 - DNA, 73 bp, Artificial Sequence
  gH29/30-rpsL-neo_For
tcgtgggggttattcttttgggcgttgcgtggggtcaggtccacgactggggcctggtgatgatggcgggatc

SEQ ID NO: 34 - DNA, 74 bp, Artificial Sequence
  gH29/30-rpsL-neo_Rev
ttcgtgtcgcgccagtacatgcggtccatgcccaggccatccaaaaaccatcagaagaactcgtcaagaaggcg

SEQ ID NO: 35 - DNA, 22 bp, Artificial Sequence
  gH29/30-scFv_For
tcgtgggggttattcttttggg

SEQ ID NO: 36 - DNA, 21 bp, Artificial Sequence
  gH29/30_scFv_Rev
ttcgtgtcgcgccagtacatg